European Patent Specification EP 3 548 105 B1, published March 5, 2025. Title: Process for the production of a nanofibre structure and nanofibre structure so obtained. Applicant: Humana Medical. The sequence listing filed with the application follows.

SEQUENCE LISTING (35 sequences)

SEQ ID NO: 1 - protein, 16 aa, Artificial Sequence
  self-assembling peptide
AEAEAKAKAEAEAKAK

SEQ ID NO: 2 - protein, 19 aa, Artificial Sequence
  self-assembling peptide with adhesion molecule
RGDAEAEAKAKAEAEAKAK

SEQ ID NO: 3 - protein, 16 aa, Artificial Sequence
  self-assembling peptide
RADARADARADARADA

SEQ ID NO: 4 - protein, 16 aa, Artificial Sequence
  self-assembling peptide
RADARGDARADARGDA

SEQ ID NO: 5 - protein, 8 aa, Artificial Sequence
  self-assembling peptide
RADARADA

SEQ ID NO: 6 - protein, 16 aa, Artificial Sequence
  self-assembling peptide
RARADADARARADADA

SEQ ID NO: 7 - protein, 8 aa, Artificial Sequence
  self-assembling peptide
RARADADA

SEQ ID NO: 8 - protein, 16 aa, Artificial Sequence
  self-assembling peptide
AEAKAEAKAEAKAEAK

SEQ ID NO: 9 - protein, 8 aa, Artificial Sequence
  self-assembling peptide
AEAKAEAK

SEQ ID NO: 10 - protein, 16 aa, Artificial Sequence
  self-assembling peptide
RAEARAEARAEARAEA

SEQ ID NO: 11 - protein, 8 aa, Artificial Sequence
  self-assembling peptide
RAEARAEA

SEQ ID NO: 12 - protein, 16 aa, Artificial Sequence
  self-assembling peptide
KADAKADAKADAKADA

SEQ ID NO: 13 - protein, 8 aa, Artificial Sequence
  self-assembling peptide
KADAKADA

SEQ ID NO: 14 - protein, 16 aa, Artificial Sequence
  self-assembling peptide
AEAEAHAHAEAEAHAH

SEQ ID NO: 15 - protein, 8 aa, Artificial Sequence
  self-assembling peptide
AEAEAHAH

SEQ ID NO: 16 - protein, 16 aa, Artificial Sequence
  self-assembling peptide
FEFEFKFKFEFEFKFK

SEQ ID NO: 17 - protein, 12 aa, Artificial Sequence
  self-assembling peptide
FEFKFEFKFEFK

SEQ ID NO: 18 - protein, 8 aa, Artificial Sequence
  self-assembling peptide
FEFKFEFK

SEQ ID NO: 19 - protein, 16 aa, Artificial Sequence
  self-assembling peptide
LELELKLKLELELKLK

SEQ ID NO: 20 - protein, 8 aa, Artificial Sequence
  self-assembling peptide
LELELKLK

SEQ ID NO: 21 - protein, 12 aa, Artificial Sequence
  self-assembling peptide
AEAEAEAEAKAK

SEQ ID NO: 22 - protein, 8 aa, Artificial Sequence
  self-assembling peptide
AEAEAKAK

SEQ ID NO: 23 - protein, 16 aa, Artificial Sequence
  self-assembling peptide
KAKAKAKAEAEAEAEA

SEQ ID NO: 24 - protein, 16 aa, Artificial Sequence
  self-assembling peptide
AEAEAEAEAKAKAKAK

SEQ ID NO: 25 - protein, 12 aa, Artificial Sequence
  self-assembling peptide
KLDLKLDLKLDL

SEQ ID NO: 26 - protein, 12 aa, Artificial Sequence
  self-assembling peptide
KLELKLELKLEL

SEQ ID NO: 27 - protein, 16 aa, Artificial Sequence
  self-assembling peptide
RARARARADADADADA

SEQ ID NO: 28 - protein, 16 aa, Artificial Sequence
  self-assembling peptide
DADADADARARARARA

SEQ ID NO: 29 - protein, 16 aa, Artificial Sequence
  self-assembling peptide
ADADADADARARARAR

SEQ ID NO: 30 - protein, 32 aa, Artificial Sequence
  self-assembling peptide
ADADADADARARARARADADADADARARARAR

SEQ ID NO: 31 - protein, 16 aa, Artificial Sequence
  self-assembling peptide
HEHEHKHKHEHEHKHK

SEQ ID NO: 32 - protein, 8 aa, Artificial Sequence
  self-assembling peptide
HEHEHKHK

SEQ ID NO: 33 - protein, 20 aa, Artificial Sequence
  self-assembling peptide
VEVEVEVEVEVEVEVEVEVE

SEQ ID NO: 34 - protein, 20 aa, Artificial Sequence
  self-assembling peptide
RFRFRFRFRFRFRFRFRFRF

SEQ ID NO: 35 - protein, 5 aa, Artificial Sequence
  adhesion peptide
PHSRN